European Patent Specification EP 3 349 788 B1, published April 9, 2025. Title: ANTI-MALARIA COMPOSITIONS AND METHODS. Applicant: ARTIFICIAL CELL TECHNOLOGIES, INC. The sequence listing filed with the application follows.

SEQUENCE LISTING (17 sequences)

SEQ ID NO: 1 - protein, 16 aa, Plasmodium falciparum
DPNANPNVDPNANPNV

SEQ ID NO: 2 - protein, 12 aa, Plasmodium falciparum
NANPNANPNANP

SEQ ID NO: 3 - protein, 20 aa, Plasmodium falciparum
EYLNKIQNSLSTEWSPCSVT

SEQ ID NO: 4 - protein, 48 aa, Plasmodium falciparum
DPNANPNVDPNANPNVNANPNANPNANPEYLNKIQNSLSTEWSPCSVT

SEQ ID NO: 5 - protein, 20 aa, Artificial Sequence
  modified T* epitope
EYLNKIQNSLSTEWSPSSVT

SEQ ID NO: 6 - protein, 20 aa, Artificial
  modified T* epitope
EYLNKIQNSLSTEWSPASVT

SEQ ID NO: 7 - protein, 48 aa, Artificial Sequence
  modified T1BT* epitope
DPNANPNVDPNANPNVNANPNANPNANPEYLNKIQNSLSTEWSPSSVT

SEQ ID NO: 8 - protein, 48 aa, Artificial Sequence
  modified T1BT* epitope
DPNANPNVDPNANPNVNANPNANPNANPEYLNKIQNSLSTEWSPASVT

SEQ ID NO: 9 - protein, 20 aa, Artificial Sequence
  surface adsorption region
KKKKKKKKKKKKKKKKKKKK

SEQ ID NO: 10 - protein, 73 aa, Artificial Sequence
  designed peptide
DPNANPNVDPNANPNVNANPNANPNANPEYLNKIQNSLSTEWSPCSVTSGNGKKKKKKKKKKKKKKKKKKKKY

SEQ ID NO: 11 - protein, 84 aa, Artificial Sequence
  designed peptide
PAMCYSSKKKKDPNANPNVDPNANPNVNANPNANPNANPEYLNKIQNSLSTEWSPCSVTSGNGKKKKKKKKKKKKKKKKKKKKY

SEQ ID NO: 12 - protein, 72 aa, Artificial Sequence
  designed peptide
DPNANPNVDPNANPNVNANPNANPNANPEYLNKIQNSLSTEWSPSSVTSGNGKKKKKKKKKKKKKKKKKKKK

SEQ ID NO: 13 - protein, 83 aa, Artificial Sequence
  designed peptide
PAMCYSSKKKKDPNANPNVDPNANPNVNANPNANPNANPEYLNKIQNSLSTEWSPSSVTSGNGKKKKKKKKKKKKKKKKKKKK

SEQ ID NO: 14 - protein, 72 aa, Artificial Sequence
  designed peptide
DPNANPNVDPNANPNVNANPNANPNANPEYLNKIQNSLSTEWSPASVTSGNGKKKKKKKKKKKKKKKKKKKK

SEQ ID NO: 15 - protein, 83 aa, Artificial Sequence
  designed peptide
PAMCYSSKKKKDPNANPNVDPNANPNVNANPNANPNANPEYLNKIQNSLSTEWSPASVTSGNGKKKKKKKKKKKKKKKKKKKK

SEQ ID NO: 16 - protein, 21 aa, Artificial Sequence
  surface adsorption region
KKKKKKKKKKKKKKKKKKKKY

SEQ ID NO: 17 - protein, 77 aa, Artificial Sequence
  designed peptide
SKKKKDPNANPNVDPNANPNVNANPNANPNANPEYLNKIQNSLSTEWSPSSVTSGNGKKKKKKKKKKKKKKKKKKKK